European Patent Application EP 4 682 256 A1, published January 21, 2026. Title: composition and use thereof. Applicant: TOAGOSEI CO., LTD. The sequence listing filed with the application follows.

SEQUENCE LISTING (8 sequences)

SEQ ID NO: 1 - RNA, 19 nt, synthetic construct
  source 1..19: mol_type = other RNA
gggtccgcgccgaggaaga

SEQ ID NO: 2 - RNA, 19 nt, synthetic construct
  source 1..19: mol_type = other RNA
cgcgccgaggaagagctaa

SEQ ID NO: 3 - protein, 20 aa, synthetic construct
MWKRWLALALALVAVAWVRA

SEQ ID NO: 4 - DNA, 60 bp, synthetic construct
  source 1..60: mol_type = other DNA
atgtggaaacgctggctcgcgctcgcgctcgcgctggtggcggtcgcctgggtccgcgcc

SEQ ID NO: 5 - DNA, 21 bp, synthetic construct
  misc_feature 1..19: note = RNA
  misc_feature 20..21: note = DNA
  source 1..21: mol_type = other DNA
  modified_base 4: mod_base = OTHER; note = uracil
gggtccgcgccgaggaagatt

SEQ ID NO: 6 - DNA, 21 bp, synthetic construct
  misc_feature 1..19: note = RNA
  misc_feature 20..21: note = DNA
  source 1..21: mol_type = other DNA
  modified_base 1: mod_base = OTHER; note = uracil
  modified_base 3..4: mod_base = OTHER; note = uracil
  modified_base 7: mod_base = OTHER; note = uracil
tcttcctcggcgcggaccctt

SEQ ID NO: 7 - DNA, 21 bp, synthetic construct
  misc_feature 1..19: note = RNA
  misc_feature 20..21: note = DNA
  source 1..21: mol_type = other DNA
  modified_base 17: mod_base = OTHER; note = uracil
cgcgccgaggaagagctaatt

SEQ ID NO: 8 - DNA, 21 bp, synthetic construct
  misc_feature 1..19: note = RNA
  misc_feature 20..21: note = DNA
  source 1..21: mol_type = other DNA
  modified_base 1..2: mod_base = OTHER; note = uracil
  modified_base 6: mod_base = OTHER; note = uracil
  modified_base 8..9: mod_base = OTHER; note = uracil
  modified_base 12: mod_base = OTHER; note = uracil
ttagctcttcctcggcgcgtt